European Patent Specification EP 3 733 705 B1, published June 24, 2026. Title: Monoclonal antibodies and methods for using same. Applicant: JSC "BIOCAD". Application PCT/RU2018/050168. The sequence listing filed with the application follows.

SEQUENCE LISTING (33 sequences)

SEQ ID NO: 1 - protein, 5 aa, Artificial Sequence
  HCDR1 amino acid sequence (according to the Kabat numbering scheme)
DYLVH

SEQ ID NO: 2 - protein, 17 aa, Artificial Sequence
  HCDR2 amino acid sequence (according to the Kabat numbering scheme)
WINTYTGTPTYADDFEG

SEQ ID NO: 3 - protein, 13 aa, Artificial Sequence
  HCDR3 amino acid sequence (according to the Kabat numbering scheme)
SWRRGLRGLGFDY

SEQ ID NO: 4 - protein, 13 aa, Artificial Sequence
  HCDR3 amino acid sequence (according to the Kabat numbering scheme)
SWRRGLRGIGFDY

SEQ ID NO: 5 - protein, 13 aa, Artificial Sequence
  HCDR3 amino acid sequence (according to the Kabat numbering scheme)
SWRRGIRGLGFDY

SEQ ID NO: 6 - protein, 13 aa, Artificial Sequence
  HCDR3 amino acid sequence (according to the Kabat numbering scheme)
SWRRGIRGIGFDY

SEQ ID NO: 7 - protein, 11 aa, Artificial Sequence
  LCDR1 amino acid sequence (according to the Kabat numbering scheme)
KASKSINKYLA

SEQ ID NO: 8 - protein, 7 aa, Artificial Sequence
  LCDR2 amino acid sequence (according to the Kabat numbering scheme)
DGSTLQS

SEQ ID NO: 9 - protein, 9 aa, Artificial Sequence
  LCDR3 amino acid sequence (according to the Kabat numbering scheme)
QQHNEYPPT

SEQ ID NO: 10 - DNA, 321 bp, Artificial Sequence
  The nucleotide sequence of the antibody light chain variable domain
gacgtgcagatgacccagtccccctacaacctggccgcctcccccggcgagtccgtgtccatcaactgcaaggcctccaagtccatcaacaagtacctggcctggtaccagcagaagcccggcaagcccaacaagctgctgatctacgacggctccaccctgcagtccggcatcccctccaggttctccggctccggctccggcaccgacttcaccctgaccatcaggggcctggagcccgaggacttcggcctgtactactgccagcagcacaacgagtacccccccaccttcggcgccggcaccaagctggagctgaag

SEQ ID NO: 11 - protein, 107 aa, Artificial Sequence
  The amino acid sequence of the antibody light chain variable domain
DVQMTQSPYNLAASPGESVSINCKASKSINKYLAWYQQKPGKPNKLLIYDGSTLQSGIPSRFSGSGSGTDFTLTIRGLEPEDFGLYYCQQHNEYPPTFGAGTKLELK

SEQ ID NO: 12 - DNA, 366 bp, Artificial Sequence
  The nucleotide sequence of the antibody heavy chain variable domain
cagatccagctggtgcagtccggccccgagctgagggagcccggcgagtccgtgaagctgtcctgcaaggcctccggctacaccttcaccgactacctggtgcactgggtgaagcaggcccccggcaagggcctgaagtggatgggctggatcaacacctacaccggcacccccacctacgccgacgacttcgagggcaggttcgtgttctccctggaggcctccgcctccaccgccaacctgcagatctccaacctgaagaacgaggacaccgccacctacttctgcgccaggtcctggaggaggggcctgaggggcctgggcttcgactactggggccagggcgtgttcgtgaccgtgtcctcc

SEQ ID NO: 13 - protein, 122 aa, Artificial Sequence
  The amino acid sequence of the antibody heavy chain variable domain
QIQLVQSGPELREPGESVKLSCKASGYTFTDYLVHWVKQAPGKGLKWMGWINTYTGTPTYADDFEGRFVFSLEASASTANLQISNLKNEDTATYFCARSWRRGLRGLGFDYWGQGVFVTVSS

SEQ ID NO: 14 - DNA, 366 bp, Artificial Sequence
  The nucleotide sequence of the antibody heavy chain variable domain
cagatccagctggtgcagtccggccccgagctgagggagcccggcgagtccgtgaagctgtcctgcaaggcctccggctacaccttcaccgactacctggtgcactgggtgaagcaggcccccggcaagggcctgaagtggatgggctggatcaacacctacaccggcacccccacctacgccgacgacttcgagggcaggttcgtgttctccctggaggcctccgcctccaccgccaacctgcagatctccaacctgaagaacgaggacaccgccacctacttctgcgccaggtcctggaggaggggcctgaggggcatcggcttcgactactggggccagggcgtgttcgtgaccgtgtcctcc

SEQ ID NO: 15 - protein, 122 aa, Artificial Sequence
  The amino acid sequence of the antibody heavy chain variable domain
QIQLVQSGPELREPGESVKLSCKASGYTFTDYLVHWVKQAPGKGLKWMGWINTYTGTPTYADDFEGRFVFSLEASASTANLQISNLKNEDTATYFCARSWRRGLRGIGFDYWGQGVFVTVSS

SEQ ID NO: 16 - DNA, 366 bp, Artificial Sequence
  The nucleotide sequence of the antibody heavy chain variable domain
cagatccagctggtgcagtccggccccgagctgagggagcccggcgagtccgtgaagctgtcctgcaaggcctccggctacaccttcaccgactacctggtgcactgggtgaagcaggcccccggcaagggcctgaagtggatgggctggatcaacacctacaccggcacccccacctacgccgacgacttcgagggcaggttcgtgttctccctggaggcctccgcctccaccgccaacctgcagatctccaacctgaagaacgaggacaccgccacctacttctgcgccaggtcctggaggaggggcatcaggggcctgggcttcgactactggggccagggcgtgttcgtgaccgtgtcctcc

SEQ ID NO: 17 - protein, 122 aa, Artificial Sequence
  The amino acid sequence of the antibody heavy chain variable domain
QIQLVQSGPELREPGESVKLSCKASGYTFTDYLVHWVKQAPGKGLKWMGWINTYTGTPTYADDFEGRFVFSLEASASTANLQISNLKNEDTATYFCARSWRRGIRGLGFDYWGQGVFVTVSS

SEQ ID NO: 18 - DNA, 366 bp, Artificial Sequence
  The nucleotide sequence of the antibody heavy chain variable domain
cagatccagctggtgcagtccggccccgagctgagggagcccggcgagtccgtgaagctgtcctgcaaggcctccggctacaccttcaccgactacctggtgcactgggtgaagcaggcccccggcaagggcctgaagtggatgggctggatcaacacctacaccggcacccccacctacgccgacgacttcgagggcaggttcgtgttctccctggaggcctccgcctccaccgccaacctgcagatctccaacctgaagaacgaggacaccgccacctacttctgcgccaggtcctggaggaggggcatcaggggcatcggcttcgactactggggccagggcgtgttcgtgaccgtgtcctcc

SEQ ID NO: 19 - protein, 122 aa, Artificial Sequence
  The amino acid sequence of the antibody heavy chain variable domain
QIQLVQSGPELREPGESVKLSCKASGYTFTDYLVHWVKQAPGKGLKWMGWINTYTGTPTYADDFEGRFVFSLEASASTANLQISNLKNEDTATYFCARSWRRGIRGIGFDYWGQGVFVTVSS

SEQ ID NO: 20 - DNA, 1365 bp, Artificial Sequence
  The nucleotide sequence of the anti-TRBV9-1 antibody heavy chain
cagatccagctggtgcagtccggccccgagctgagggagcccggcgagtccgtgaagctgtcctgcaaggcctccggctacaccttcaccgactacctggtgcactgggtgaagcaggcccccggcaagggcctgaagtggatgggctggatcaacacctacaccggcacccccacctacgccgacgacttcgagggcaggttcgtgttctccctggaggcctccgcctccaccgccaacctgcagatctccaacctgaagaacgaggacaccgccacctacttctgcgccaggtcctggaggaggggcctgaggggcctgggcttcgactactggggccagggcgtgttcgtgaccgtgtcctccgcctccaccaagggcccatcggtcttccccctggcaccctcctccaagagcacctctgggggcacagcggccctgggctgcctggtcaaggactacttccccgaaccggtgacggtgtcgtggaactcaggcgccctgaccagcggcgtgcacaccttcccggctgtcctacagtcctcaggactctactccctcagcagcgtggtgactgtgccctctagcagcttgggcacccagacctacatctgcaacgtgaatcacaagcccagcaacaccaaggtggacaagaaagttgagcccccgaaatcttgtgacaaaactcacacatgcccaccgtgcccagcacctgaactcctggggggaccgtcagtcttcctcttccccccaaaacccaaggacaccctcatgatctcccggacccctgaggtcacatgcgtggtggtggacgtgagccacgaagaccctgaggtcaagttcaactggtacgtggacggcgtggaggtgcataatgccaagacaaagccgcgggaggagcagtacaacagcacgtaccgtgtggtcagcgtcctcaccgtcctgcaccaggactggctgaatggcaaggagtacaagtgcaaggtctccaacaaagccctcccagcccccatcgagaaaaccatctccaaagccaaagggcagccccgagaaccacaggtgtacaccctgcccccatcccgggatgagctgaccaagaaccaggtcagcctgacctgcctggtcaaaggcttctatcccagcgacatcgccgtggagtgggagagcaatgggcagccggagaacaactacaagaccacgcctcccgtgctggactccgacggctccttcttcctctacagcaagctcaccgtggacaagagcaggtggcagcaggggaacgtcttctcatgctccgtgatgcatgaggctctgcacaaccactacacgcagaagagcctctccctgtctccgggtaaatgataa

SEQ ID NO: 21 - protein, 452 aa, Artificial Sequence
  The amino acid sequence of the anti-TRBV9-1 antibody heavy chain
QIQLVQSGPELREPGESVKLSCKASGYTFTDYLVHWVKQAPGKGLKWMGWINTYTGTPTYADDFEGRFVFSLEASASTANLQISNLKNEDTATYFCARSWRRGLRGLGFDYWGQGVFVTVSSASTKGPSVFPLAPSSKSTSGGTAALGCLVKDYFPEPVTVSWNSGALTSGVHTFPAVLQSSGLYSLSSVVTVPSSSLGTQTYICNVNHKPSNTKVDKKVEPKSCDKTHTCPPCPAPELLGGPSVFLFPPKPKDTLMISRTPEVTCVVVDVSHEDPEVKFNWYVDGVEVHNAKTKPREEQYNSTYRVVSVLTVLHQDWLNGKEYKCKVSNKALPAPIEKTISKAKGQPREPQVYTLPPSRDELTKNQVSLTCLVKGFYPSDIAVEWESNGQPENNYKTTPPVLDSDGSFFLYSKLTVDKSRWQQGNVFSCSVMHEALHNHYTQKSLSLSPGK

SEQ ID NO: 22 - DNA, 1365 bp, Artificial Sequence
  The nucleotide sequence of the anti-TRBV9-2 antibody heavy chain
cagatccagctggtgcagtccggccccgagctgagggagcccggcgagtccgtgaagctgtcctgcaaggcctccggctacaccttcaccgactacctggtgcactgggtgaagcaggcccccggcaagggcctgaagtggatgggctggatcaacacctacaccggcacccccacctacgccgacgacttcgagggcaggttcgtgttctccctggaggcctccgcctccaccgccaacctgcagatctccaacctgaagaacgaggacaccgccacctacttctgcgccaggtcctggaggaggggcctgaggggcatcggcttcgactactggggccagggcgtgttcgtgaccgtgtcctccgcctccaccaagggcccatcggtcttccccctggcaccctcctccaagagcacctctgggggcacagcggccctgggctgcctggtcaaggactacttccccgaaccggtgacggtgtcgtggaactcaggcgccctgaccagcggcgtgcacaccttcccggctgtcctacagtcctcaggactctactccctcagcagcgtggtgactgtgccctctagcagcttgggcacccagacctacatctgcaacgtgaatcacaagcccagcaacaccaaggtggacaagaaagttgagcccccgaaatcttgtgacaaaactcacacatgcccaccgtgcccagcacctgaactcctggggggaccgtcagtcttcctcttccccccaaaacccaaggacaccctcatgatctcccggacccctgaggtcacatgcgtggtggtggacgtgagccacgaagaccctgaggtcaagttcaactggtacgtggacggcgtggaggtgcataatgccaagacaaagccgcgggaggagcagtacaacagcacgtaccgtgtggtcagcgtcctcaccgtcctgcaccaggactggctgaatggcaaggagtacaagtgcaaggtctccaacaaagccctcccagcccccatcgagaaaaccatctccaaagccaaagggcagccccgagaaccacaggtgtacaccctgcccccatcccgggatgagctgaccaagaaccaggtcagcctgacctgcctggtcaaaggcttctatcccagcgacatcgccgtggagtgggagagcaatgggcagccggagaacaactacaagaccacgcctcccgtgctggactccgacggctccttcttcctctacagcaagctcaccgtggacaagagcaggtggcagcaggggaacgtcttctcatgctccgtgatgcatgaggctctgcacaaccactacacgcagaagagcctctccctgtctccgggtaaatgataa

SEQ ID NO: 23 - protein, 452 aa, Artificial Sequence
  The amino acid sequence of the anti-TRBV9-2 antibody heavy chain
QIQLVQSGPELREPGESVKLSCKASGYTFTDYLVHWVKQAPGKGLKWMGWINTYTGTPTYADDFEGRFVFSLEASASTANLQISNLKNEDTATYFCARSWRRGLRGIGFDYWGQGVFVTVSSASTKGPSVFPLAPSSKSTSGGTAALGCLVKDYFPEPVTVSWNSGALTSGVHTFPAVLQSSGLYSLSSVVTVPSSSLGTQTYICNVNHKPSNTKVDKKVEPKSCDKTHTCPPCPAPELLGGPSVFLFPPKPKDTLMISRTPEVTCVVVDVSHEDPEVKFNWYVDGVEVHNAKTKPREEQYNSTYRVVSVLTVLHQDWLNGKEYKCKVSNKALPAPIEKTISKAKGQPREPQVYTLPPSRDELTKNQVSLTCLVKGFYPSDIAVEWESNGQPENNYKTTPPVLDSDGSFFLYSKLTVDKSRWQQGNVFSCSVMHEALHNHYTQKSLSLSPGK

SEQ ID NO: 24 - DNA, 1365 bp, Artificial Sequence
  The nucleotide sequence of the anti-TRBV9-3 antibody heavy chain
cagatccagctggtgcagtccggccccgagctgagggagcccggcgagtccgtgaagctgtcctgcaaggcctccggctacaccttcaccgactacctggtgcactgggtgaagcaggcccccggcaagggcctgaagtggatgggctggatcaacacctacaccggcacccccacctacgccgacgacttcgagggcaggttcgtgttctccctggaggcctccgcctccaccgccaacctgcagatctccaacctgaagaacgaggacaccgccacctacttctgcgccaggtcctggaggaggggcatcaggggcctgggcttcgactactggggccagggcgtgttcgtgaccgtgtcctccgcctccaccaagggcccatcggtcttccccctggcaccctcctccaagagcacctctgggggcacagcggccctgggctgcctggtcaaggactacttccccgaaccggtgacggtgtcgtggaactcaggcgccctgaccagcggcgtgcacaccttcccggctgtcctacagtcctcaggactctactccctcagcagcgtggtgactgtgccctctagcagcttgggcacccagacctacatctgcaacgtgaatcacaagcccagcaacaccaaggtggacaagaaagttgagcccccgaaatcttgtgacaaaactcacacatgcccaccgtgcccagcacctgaactcctggggggaccgtcagtcttcctcttccccccaaaacccaaggacaccctcatgatctcccggacccctgaggtcacatgcgtggtggtggacgtgagccacgaagaccctgaggtcaagttcaactggtacgtggacggcgtggaggtgcataatgccaagacaaagccgcgggaggagcagtacaacagcacgtaccgtgtggtcagcgtcctcaccgtcctgcaccaggactggctgaatggcaaggagtacaagtgcaaggtctccaacaaagccctcccagcccccatcgagaaaaccatctccaaagccaaagggcagccccgagaaccacaggtgtacaccctgcccccatcccgggatgagctgaccaagaaccaggtcagcctgacctgcctggtcaaaggcttctatcccagcgacatcgccgtggagtgggagagcaatgggcagccggagaacaactacaagaccacgcctcccgtgctggactccgacggctccttcttcctctacagcaagctcaccgtggacaagagcaggtggcagcaggggaacgtcttctcatgctccgtgatgcatgaggctctgcacaaccactacacgcagaagagcctctccctgtctccgggtaaatgataa

SEQ ID NO: 25 - protein, 452 aa, Artificial Sequence
  The amino acid sequence of the anti-TRBV9-3 antibody heavy chain
QIQLVQSGPELREPGESVKLSCKASGYTFTDYLVHWVKQAPGKGLKWMGWINTYTGTPTYADDFEGRFVFSLEASASTANLQISNLKNEDTATYFCARSWRRGIRGLGFDYWGQGVFVTVSSASTKGPSVFPLAPSSKSTSGGTAALGCLVKDYFPEPVTVSWNSGALTSGVHTFPAVLQSSGLYSLSSVVTVPSSSLGTQTYICNVNHKPSNTKVDKKVEPKSCDKTHTCPPCPAPELLGGPSVFLFPPKPKDTLMISRTPEVTCVVVDVSHEDPEVKFNWYVDGVEVHNAKTKPREEQYNSTYRVVSVLTVLHQDWLNGKEYKCKVSNKALPAPIEKTISKAKGQPREPQVYTLPPSRDELTKNQVSLTCLVKGFYPSDIAVEWESNGQPENNYKTTPPVLDSDGSFFLYSKLTVDKSRWQQGNVFSCSVMHEALHNHYTQKSLSLSPGK

SEQ ID NO: 26 - DNA, 1365 bp, Artificial Sequence
  The nucleotide sequence of the anti-TRBV9-4 antibody heavy chain
cagatccagctggtgcagtccggccccgagctgagggagcccggcgagtccgtgaagctgtcctgcaaggcctccggctacaccttcaccgactacctggtgcactgggtgaagcaggcccccggcaagggcctgaagtggatgggctggatcaacacctacaccggcacccccacctacgccgacgacttcgagggcaggttcgtgttctccctggaggcctccgcctccaccgccaacctgcagatctccaacctgaagaacgaggacaccgccacctacttctgcgccaggtcctggaggaggggcatcaggggcatcggcttcgactactggggccagggcgtgttcgtgaccgtgtcctccgcctccaccaagggcccatcggtcttccccctggcaccctcctccaagagcacctctgggggcacagcggccctgggctgcctggtcaaggactacttccccgaaccggtgacggtgtcgtggaactcaggcgccctgaccagcggcgtgcacaccttcccggctgtcctacagtcctcaggactctactccctcagcagcgtggtgactgtgccctctagcagcttgggcacccagacctacatctgcaacgtgaatcacaagcccagcaacaccaaggtggacaagaaagttgagcccccgaaatcttgtgacaaaactcacacatgcccaccgtgcccagcacctgaactcctggggggaccgtcagtcttcctcttccccccaaaacccaaggacaccctcatgatctcccggacccctgaggtcacatgcgtggtggtggacgtgagccacgaagaccctgaggtcaagttcaactggtacgtggacggcgtggaggtgcataatgccaagacaaagccgcgggaggagcagtacaacagcacgtaccgtgtggtcagcgtcctcaccgtcctgcaccaggactggctgaatggcaaggagtacaagtgcaaggtctccaacaaagccctcccagcccccatcgagaaaaccatctccaaagccaaagggcagccccgagaaccacaggtgtacaccctgcccccatcccgggatgagctgaccaagaaccaggtcagcctgacctgcctggtcaaaggcttctatcccagcgacatcgccgtggagtgggagagcaatgggcagccggagaacaactacaagaccacgcctcccgtgctggactccgacggctccttcttcctctacagcaagctcaccgtggacaagagcaggtggcagcaggggaacgtcttctcatgctccgtgatgcatgaggctctgcacaaccactacacgcagaagagcctctccctgtctccgggtaaatgataa

SEQ ID NO: 27 - protein, 452 aa, Artificial Sequence
  The amino acid sequence of the anti-TRBV9-4 antibody heavy chain
QIQLVQSGPELREPGESVKLSCKASGYTFTDYLVHWVKQAPGKGLKWMGWINTYTGTPTYADDFEGRFVFSLEASASTANLQISNLKNEDTATYFCARSWRRGIRGIGFDYWGQGVFVTVSSASTKGPSVFPLAPSSKSTSGGTAALGCLVKDYFPEPVTVSWNSGALTSGVHTFPAVLQSSGLYSLSSVVTVPSSSLGTQTYICNVNHKPSNTKVDKKVEPKSCDKTHTCPPCPAPELLGGPSVFLFPPKPKDTLMISRTPEVTCVVVDVSHEDPEVKFNWYVDGVEVHNAKTKPREEQYNSTYRVVSVLTVLHQDWLNGKEYKCKVSNKALPAPIEKTISKAKGQPREPQVYTLPPSRDELTKNQVSLTCLVKGFYPSDIAVEWESNGQPENNYKTTPPVLDSDGSFFLYSKLTVDKSRWQQGNVFSCSVMHEALHNHYTQKSLSLSPGK

SEQ ID NO: 28 - DNA, 639 bp, Artificial Sequence
  The nucleotide sequence of the anti-TRBV9 antibody light chain
gacgtgcagatgacccagtccccctacaacctggccgcctcccccggcgagtccgtgtccatcaactgcaaggcctccaagtccatcaacaagtacctggcctggtaccagcagaagcccggcaagcccaacaagctgctgatctacgacggctccaccctgcagtccggcatcccctccaggttctccggctccggctccggcaccgacttcaccctgaccatcaggggcctggagcccgaggacttcggcctgtactactgccagcagcacaacgagtacccccccaccttcggcgccggcaccaagctggagctgaagcgaactgtggctgcaccatctgtcttcatcttcccgccatctgatgagcagttgaaatctggaactgcctctgtcgtgtgcctgctgaataacttctatcccagagaggccaaagtacagtggaaggtggataacgccctccaatcgggtaactcccaggagagtgtcacagagcaggacagcaaggacagcacctacagcctcagcagcaccctgacgctgagcaaagcagactacgagaaacacaaagtctacgcctgcgaagtcacccatcagggcctgtcctcgcccgtcacaaagagcttcaacaggggagag

SEQ ID NO: 29 - protein, 214 aa, Artificial Sequence
  The amino acid sequence of the anti-TRBV9 antibody light chain
DVQMTQSPYNLAASPGESVSINCKASKSINKYLAWYQQKPGKPNKLLIYDGSTLQSGIPSRFSGSGSGTDFTLTIRGLEPEDFGLYYCQQHNEYPPTFGAGTKLELKRTVAAPSVFIFPPSDEQLKSGTASVVCLLNNFYPREAKVQWKVDNALQSGNSQESVTEQDSKDSTYSLSSTLTLSKADYEKHKVYACEVTHQGLSSPVTKSFNRGEC

SEQ ID NO: 30 - DNA, 333 bp, Artificial Sequence
  The nucleotide sequence of the variant of the antibody heavy chain variable domain
cagatccagttggtgcagtccggccccgagctgaaggagcccggcgagtccgtgaagatctcctgcaaggcctccggctacaccttcaccgactacctggtgcactgggtgaagcaggcccccggcaagggcatcaagtggatgggctggatcaacacctacaccggcacccccacctacgccgacgacttcgagggcaggttcgtgttctccatcgaggcctccgcctccaccgccaacctgcagatctccaacatcaagaacgaggacaccgccacctacttctgcgccaggtcctggaggaggggcctgaggggcctgggcttcgactac

SEQ ID NO: 31 - protein, 111 aa, Artificial Sequence
  The amino acid sequence of the variant of the antibody heavy chain variable domain
QIQLVQSGPELKEPGESVKISCKASGYTFTDYLVHWVKQAPGKGIKWMGWINTYTGTPTYADDFEGRFVFSIEASASTANLQISNIKNEDTATYFCARSWRRGLRGLGFDY

SEQ ID NO: 32 - DNA, 333 bp, Artificial Sequence
  The nucleotide sequence of the variant of the antibody heavy chain variable domain
cagatccagttggtgcagtccggccccgagataaaggagcccggcgagtccgtgaagatctcctgcaaggcctccggctacaccttcaccgactacctggtgcactgggtgaagcaggcccccggcaagggcatcaagtggatgggctggatcaacacctacaccggcacccccacctacgccgacgacttcgagggcaggttcgtgttctccatcgaggcctccgcctccaccgccaacctgcagatctccaacatcaagaacgaggacaccgccacctacttctgcgccaggtcctggaggaggggcctgaggggcctgggcttcgactac

SEQ ID NO: 33 - protein, 111 aa, Artificial Sequence
  The amino acid sequence of the variant of the antibody heavy chain variable domain
QIQLVQSGPEIKEPGESVKISCKASGYTFTDYLVHWVKQAPGKGIKWMGWINTYTGTPTYADDFEGRFVFSIEASASTANLQISNIKNEDTATYFCARSWRRGLRGLGFDY